European Patent Application EP 4 775 674 A1, published July 15, 2026. Title: ガイドＲＮＡおよびその利用. Applicant: C4U Corporation. The sequence listing filed with the application follows.

SEQUENCE LISTING (18 sequences)

SEQ ID NO: 1 - DNA, 30 bp, Pyrococcus furiosus
  source 1..30: mol_type = genomic DNA
gttccaataagactacaaaagaattgaaag

SEQ ID NO: 2 - DNA, 36 bp, Synechocystis sp.
  source 1..36: mol_type = genomic DNA
gtgtccaaaccattgatgccgtaaggcgttgagcac

SEQ ID NO: 3 - DNA, 32 bp, Neisseria lactamica
  source 1..32: mol_type = genomic DNA
tcagccgcctctaggcggctgtgtgttgaaac

SEQ ID NO: 4 - DNA, 37 bp, Microcystis aeruginosa
  source 1..37: mol_type = genomic DNA
gttccaattaatcttaagccctattagggattgaaac

SEQ ID NO: 5 - DNA, 29 bp, Escherichia coli
  source 1..29: mol_type = genomic DNA
gtgttccccgcgccagcggggataaaccg

SEQ ID NO: 6 - DNA, 28 bp, Pseudomonas aeruginosa
  source 1..28: mol_type = genomic DNA
gttcactgccgtataggcagctaagaaa

SEQ ID NO: 7 - DNA, 36 bp, Thioalkalivibrio sulfidiphilus
  source 1..36: mol_type = genomic DNA
gtcatccgcggcatttagccgcggcctcattgaagc

SEQ ID NO: 8 - RNA, 90 nt, synthetic construct
  source 1..90: mol_type = other RNA
gtgttccccgcgccagcggggataaaccgggacacactgcttgggggctctgaaatatggagtgttccccgcgccagcggggataaaccg

SEQ ID NO: 9 - RNA, 61 nt, synthetic construct
  source 1..61: mol_type = other RNA
ataaaccgggacacactgcttgggggctctgaaatatggagtgttccccgcgccagcgggg

SEQ ID NO: 10 - DNA, 16 bp, synthetic construct
  source 1..16: mol_type = other DNA
gtcaacggatttggtc

SEQ ID NO: 11 - DNA, 60 bp, Mus musculus
  source 1..60: mol_type = other DNA
gcattactatgtgtcaagggacacactgcttgggggctctgaaatatggagggacattga

SEQ ID NO: 12 - RNA, 61 nt, synthetic construct
  source 1..61: mol_type = other RNA
gtgttccccgcgccagcggggataaaccgggacacactgcttgggggctctgaaatatgga

SEQ ID NO: 13 - RNA, 90 nt, synthetic construct
  source 1..90: mol_type = other RNA
gtgttccccgcgccagcggggataaaccgcaggccaatggggaggacatcgatgtcacctcgtgttccccgcgccagcggggataaaccg

SEQ ID NO: 14 - RNA, 61 nt, synthetic construct
  source 1..61: mol_type = other RNA
gtgttccccgcgccagcggggataaaccgcaggccaatggggaggacatcgatgtcacctc

SEQ ID NO: 15 - RNA, 98 nt, synthetic construct
  source 1..98: mol_type = other RNA
tcagccgcctctaggcggctgtgtgttgaaaccagaaccggaggacaaagtacaaacggcagaagctcagccgcctctaggcggctgtgtgttgaaac

SEQ ID NO: 16 - RNA, 66 nt, synthetic construct
  source 1..66: mol_type = other RNA
tcagccgcctctaggcggctgtgtgttgaaaccagaaccggaggacaaagtacaaacggcagaagc

SEQ ID NO: 17 - RNA, 109 nt, synthetic construct
  source 1..109: mol_type = other RNA
gttccaattaatcttaagccctattagggattgaaacccagaaccggaggacaaagtacaaacggcagaagcgttccaattaatcttaagccctattagggattgaaac

SEQ ID NO: 18 - RNA, 72 nt, synthetic construct
  source 1..72: mol_type = other RNA
gttccaattaatcttaagccctattagggattgaaacccagaaccggaggacaaagtacaaacggcagaagc